European Patent Specification EP 4 017 515 B1, published June 25, 2025. Title: Yeast having improvement of lactic acid tolerance and use thereof. Applicant: PTT Global Chemical Public Company Limited. Application PCT/TH2019/000030. The sequence listing filed with the application follows.

SEQUENCE LISTING (2 sequences)

SEQ ID NO: 1 - DNA, 6319 bp, Artificial Sequence
  pHAA1del2 Plasmid
gttgacagtaagacgggtaagcctgttgatgataccgctgccttactgggtgcattagccagtctgaatgacctgtcacgggataatccgaagtggtcagactggaaaatcagagggcaggaactgctgaacagcaaaaagtcagatagcaccacatagcagacccgccataaaacgccctgagaagcccgtgacgggcttttcttgtattatgggtagtttccttgcatgaatccataaaaggcgcctgtagtgccatttacccccattcactgccagagccgtgagcgcagcgaactgaatgtcacgaaaaagacagcgactcaggtgcctgatggtcggagacaaaaggaatattcagcgatttgcccgagcttgcgagggtgctacttaagcctttagggttttaaggtctgttttgtagaggagcaaacagcgtttgcgacatccttttgtaatactgcggaactgactaaagtagtgagttatacacagggctgggatctattctttttatctttttttattctttctttattctataaattataaccacttgaatataaacaaaaaaaacacacaaaggtctagcggaatttacagagggtctagcagaatttacaagttttccagcaaaggtctagcagaatttacagatacccacaactcaaaggaaaaggactagtaattatcattgactagcccatctcaattggtatagtgattaaaatcacctagaccaattgagatgtatgtctgaattagttgttttcaaagcaaatgaactagcgattagtcgctatgacttaacggagcatgaaaccaagctaattttatgctgtgtggcactactcaaccccacgattgaaaaccctacaaggaaagaacggacggtatcgttcacttataaccaatacgctcagatgatgaacatcagtagggaaaatgcttatggtgtattagctaaagcaaccagagagctgatgacgagaactgtggaaatcaggaatcctttggttaaaggctttgagattttccagtggacaaactatgccaagttctcaagcgaaaaattagaattagtttttagtgaagagatattgccttatcttttccagttaaaaaaattcataaaatataatctggaacatgttaagtcttttgaaaacaaatactctatgaggatttatgagtggttattaaaagaactaacacaaaagaaaactcacaaggcaaatatagagattagccttgatgaatttaagttcatgttaatgcttgaaaataactaccatgagtttaaaaggcttaaccaatgggttttgaaaccaataagtaaagatttaaacacttacagcaatatgaaattggtggttgataagcgaggccgcccgactgatacgttgattttccaagttgaactagatagacaaatggatctcgtaaccgaacttgagaacaaccagataaaaatgaatggtgacaaaataccaacaaccattacatcagattcctacctacgtaacggactaagaaaaacactacacgatgctttaactgcaaaaattcagctcaccagttttgaggcaaaatttttgagtgacatgcaaagtaagcatgatctcaatggttcgttctcatggctcacgcaaaaacaacgaaccacactagagaacatactggctaaatacggaaggatctgaggttcttatggccattagccatcatcgtatccgatattcaagtatcatcacacttaccaacacaattatttttttttttttttattttaaatattaagaaaagagagaataaagaagaagtggtaaaagacaaacaaggagcaagcgtttagtggggatctaacaaacaacacaacaacaacatactctgtgctttgaagtgtaaactactatatcattatcattaatttttggatattggattttggttttttttttctgtcgagaacctctcattacttgggctttaatttaaagtcataaattattcgttttatttcatttcatttcattttattttattttaatattgggaaatttactctctcaatagtgtgtgcttttaaaaaccgggttccaaaataggttttagcgcacagatacgggttctggggaaacaccagcagcagcagtagcgaaagttttccaccgtctccagccttcttcctggtcatttttttcgatacaagccaacttaataacaaatatatatatgtgttatctatttctacctaattaaatcggtacaatccgttattgaatgtaatagttctaattatatttgttagcacgtctttcattttttcccccaaatgctctatatatattcttactctcgctactatattttatataataagagactaatcgataatatcaaattttaaattatacttgttgttacccatctatatacactgaaccctatccgagagcacataggtgtatgacaatccggtatcaaaccattcaatgggagatatactggaaaacaaaacttatatctttgtagttgtgctcattctttagtagatggtcattggtttttgccaatgcactgtgatccaaatggttccacgaggtagcatcaccatacaacattacaggcgcttttatcatttgtttaccatttttgcaacgcttacagttgtatgtctcgttcaattcatcattttttttttattcttttttttgatttcggtttctttgaaatttttttgattcggtaatctccgaacagaaggaagaacgaaggaaggagcacagacttagattggtatatatacgcatatgtagtgttgaagaaacatgaaattgcccagtattcttaacccaactgcacagaacaaaaacctgcaggaaacgaagataaatcatgtcgaaagctacatataaggaacgtgctgctactcatcctagtcctgttgctgccaagctatttaatatcatgcacgaaaagcaaacaaacttgtgtgcttcattggatgttcgtaccaccaaggaattactggagttagttgaagcattaggtcccaaaatttgtttactaaaaacacatgtggatatcttgactgatttttccatggagggcacagttaagccgctaaaggcattatccgccaagtacaattttttactcttcgaagacagaaaatttgctgacattggtaatacagtcaaattgcagtactctgcgggtgtatacagaatagcagaatgggcagacattacgaatgcacacggtgtggtgggcccaggtattgttagcggtttgaagcaggcggcagaagaagtaacaaaggaacctagaggccttttgatgttagcagaattgtcatgcaagggctccctatctactggagaatatactaagggtactgttgacattgcgaagagcgacaaagattttgttatcggctttattgctcaaagagacatgggtggaagagatgaaggttacgattggttgattatgacacccggtgtgggtttagatgacaagggagacgcattgggtcaacagtatagaaccgtggatgatgtggtctctacaggatctgacattattattgttggaagaggactatttgcaaagggaagggatgctaaggtagagggtgaacgttacagaaaagcaggctgggaagcatatttgagaagatgcggccagcaaaactaaaaaactgtattataagtaaatgcatgtatactaaactcacaaattagagcttcaatttaattatatcagttattacccgggaatctcggtcgtaatgatttttataatgacgaaaaaaaaaaaattggaaagaaaaagcttggacacaagtaaaaacacagtcgggcttgaaccgctaagtataatgaaacccatcactccaaatactagaacaaaggttggtgaagtctatatcccactaacagagtacgtcccaacaagtataacgtcttctcacgaccaaacagacagcatcaacccacttctcatgggcgacagcctgtccatatatgacgatggccagtctgatactcctaatgtaacatacttcgctgatacttctaaaagtatgtcgtatacccagttgaaggaacagcggaagtctgtcaacaatgaacacgttccttcacaaagagtgcctctagccaacactggtcgctcctcttcctttatctctaatatatcatctcatgactccgtaatctcgaataacgatttcataagttcgatgaacagttcggattctctttcgtcgatgctgcaaggtggtaacgctcaccattaccaggatatgctccatcaccccagcaatggcagaggcatggacataagcctgttcggttcgtaagctgtaatgcaagtagcgtatgcgctcacgcaactggtccagaaccttgaccgaacgcagcggtggtaacggcgcagtggcggttttcatggcttgttatgactgtttttttggggtacagtctatgcctcgggcatccaagcagcaagcgcgttacgccgtgggtcgatgtttgatgttatggagcagcaacgatgttacgcagcagggcagtcgccctaaaacaaagttaaacatcatgagggaagcggtgatcgccgaagtatcgactcaactatcagaggtagttggcgtcatcgagcgccatctcgaaccgacgttgctggccgtacatttgtacggctccgcagtggatggcggcctgaagccacacagtgatattgatttgctggttacggtgaccgtaaggcttgatgaaacaacgcggcgagctttgatcaacgaccttttggaaacttcggcttcccctggagagagcgagattctccgcgctgtagaagtcaccattgttgtgcacgacgacatcattccgtggcgttatccagctaagcgcgaactgcaatttggagaatggcagcgcaatgacattcttgcaggtatcttcgagccagccacgatcgacattgatctggctatcttgctgacaaaagcaagagaacatagcgttgccttggtaggtccagcggcggaggaactctttgatccggttcctgaacaggatctatttgaggcgctaaatgaaaccttaacgctatggaactcgccgcccgactgggctggcgatgagcgaaatgtagtgcttacgttgtcccgcatttggtacagcgcagtaaccggcaaaatcgcgccgaaggatgtcgctgccgactgggcaatggagcgcctgccggcccagtatcagcccgtcatacttgaagctagacaggcttatcttggacaagaagaagatcgcttggcctcgcgcgcagatcagttggaagaatttgtccactacgtgaaaggcgagatcaccaaggtagtcggcaaataatgtctaacaattcgttcaagccgacgccgcttcgcggcgcggcttaactcaagcgttagatgcactaagcacataattgctcacagccaaactatcaggtcaagtctgcttttattatttttaagcgtgcataataagccctacacaaattgggagatatatcatgaaaggctggctttttcttgttatcgcaatagttggcgaagtaatcgcaacatccgcattaaaatctagcgagggctttactaagctgatccggtggatgaccttttgaatgacctttaatagattatattactaattaattggggaccctagaggtccccttttttattttaaaaattttttcacaaaacggtttacaagcatacgttggccgattcattaatgcagctggcacgacaggtttcccgactggaaagcgggcagtgagcgcaacgcaattaatgtgagttagctcactcattaggcaccccaggctttacactttatgcttccggctcgtatgttgtgtggaattgtgagcggataacaatttcacacaggaaacagctatgaccatgattacgccaagcttgcatgcctgcaggtcgactctagaggatccccgggtaccgagctcgaattcactggccgtcgttttacaacgtcgtgactgggaaaaccctggcgttacccaacttaatcgccttgcagcacatccccctttcgccagctggcgtaatagcgaagaggcccgcaccgatcgcccttcccaacagttgcgcagcctgaatggcgaatggcgcctgatgcggtattttctccttacgcatctgtgcggtatttcacaccgcatatggtgcactctcagtacaatctgctctgatgccgcatagttaagccagccccgacacccgccaacacccgctgacgaattc

SEQ ID NO: 2 - protein, 599 aa, Kluyveromyces marxianus
MVLINGVKYACERCIRGHRVTTCNHTDQPLTMIKPKGRPSTTCAHCKELRKSKNANPSGQCTCGRQDKKRLAQKVKEEASCTCKTDPDHCACHKKRGAKRKTKGQNSGTSIGLDLDGKVSKSNGYSFQSLPSINSSQSLDKDISNLLGSPISMNTSFSTGWDTGSISSSNRSPPGSGNTYSNISNGNTGTISNNNNNNNNNHHHHHKHGQDTSKNTVGLEPLSIMKPITPNTRTKVGEVYIPLTEYVPTSITSSHDQTDSINPLLMGDSLSIYDDGQSDTPNVTYFADTSKSMSYTQLKEQRKSVNNEHVPSQRVPLANTGRSSSFISNISSHDSVISNNDFISSMNSSDSLSSMLQGGNAHHYQDMLHHPSNGRGSGFNPVHIEQSPNVYGFDTDSVRSVEVLSITPSFMDIPESKQASAESNTSSSGYISWKGVNSRRERSVSIHKNHRYDSENKRKRHPLTSANSSKQQIKSMILPIEENNNHNSSSSNENTAATLPTTSNNFNSPADSTNTALSSKAAFGDQSVFSTERRGLEPSFVDPQFSPDFNPSLKQSHMINQNIIDNNSLFSGTSEGNNPSPNDIFPVEFADIDDLMTHL